European Patent Specification EP 3 302 540 B1, published January 7, 2026. Title: ADENO-ASSOCIATED VIRUS MEDIATED DELIVERY OF C1EI AS A THERAPY FOR ANGIOEDEMA. Applicant: Cornell University. The sequence listing filed with the application follows.

SEQUENCE LISTING (4 sequences)

SEQ ID NO: 1 - protein, 500 aa, Artificial Sequence
  Synthetic AAM21515.1 (C1EI AA sequence)
MASRLTLLTLLLLLLAGDRASSNPNATSSSSQDPESLQDRGEGKVATTVISKMLFVEPILEVSSLPTTNSTTNSATKITANTTDEPTTQPTTEPTTQPTIQPTQPTTQLPTDSPTQPTTGSFCPGPVTLCSDLESHSTEAVLGDALVDFSLKLYHAFSAMKKVETNMAFSPFSIASLLTQVLLGAGENTKTNLESILSYPKDFTCVHQALKGFTTKGVTSVSQIFHSPDLAIRDTFVNASRTLYSSSPRVLSNNSDANLELINTWVAKNTNNKISRLLDSLPSDTRLVLLNAIYLSAKWKTTFDPKKTRMEPFHFKNSVIKVPMMNSKKYPVAHFIDQTLKAKVGQLQLSHNLSLVILVPQNLKHRLEDMEQALSPSVFKAIMEKLEMSKFQPTLLTLPRIKVTTSQDMLSIMEKLEFFDFSYDLNLCGLTEDPDLQVSAMQHQTVLELTETGVEAAAASAISVARTLLVFEVQQPFLFVLWDQQHKFPVFMGRVYDPRA

SEQ ID NO: 2 - DNA, 22243 bp, Artificial Sequence
  Synthetic AF435921.1 (C1EI nucl. Sequence)
gcccagatggcctccaggctgaccctgctgaccctcctgctgctgctgctggctggggtatgtggtcccttgtgggatgggggacgggggtggagacgggaggcgggatggtgcggggtgcgggcggtggctgaggattaacccttcaggctccggggaatgaggagagctcctcttgggatcattgagtgtgatccttgcacacgcactcgtagatggtggaaagagctcaggactcagacagatgcaagttctaatcttggcgggccatgtaggagctgcgcagcgtggtcctgaggacgtcacttttctcagcctactcctcctgatttataaaatgttgaataaacagatcccaccctgtccaccaagcaggcttggcaggaggatcacatagggcaaggagatgggaagcattttgtgatatcaaagcaagagtttgttgtagaaaagagctgtggggaggagaggtttggctgctgtgacacagacggtggtcccaggctagggcctgtgaagacagggaagaatggtagcaaacatacgtgggtctgggtgggggtcaatagcagtgagaggtcccagtggtctgggaggtcatggactagaaataaggctaagaagtgcaggatcccaggagaaaggtaggtaggggtgtgtgtatgtgcgtgtgtgtgtgtgtgcacgcgcaagttggtatcacatactcagcagatgatgtagttatgagcagggagtttggaatcagagaccttgttttgacccctagctgtttctcccatttctgtgagaccctggactagttaatatgtgtcggtatgagtttctctacctgtgaaatggagctaatgcgtggtttctcagtggaggatctgttgacattggggctggataattcattgctgaggggctaccctgcgcattttaggatgttttgcagtatatctctagcctctacgcactagattccggtagcatcttccctgctgtctccctgtgacaaccaaaaatgtctctggacattgccaaatatcccctgggagtcaaaattgtttcagagccgctggcctatactacttctctctccctcccttcctgcctcccttctttcctccttccctttcttcgttcccttcctaatgtgtactgtttttccacacccactaatgggttgcaacccacagtttaaaaatttactgttctaaatcaaggagcacaagttcaaatgtctgtactagccaagcaagtgagtcaaacaggtagatatttacaggaaattgcaagaacatagataaatgacaacactcagcttcactgtttggaaaacaacttcctacagggcagtaattggtcagagattacagagtccctgactatccctcatcttctgcagagcacattcctgtgcacccccaccctcaccctgtattgccccttctctgaggaattagtggtggtggttctaagacagattgctcatctgccgcactgtcagaaattactctcttgtacaggacattttccacatccacaccttctcttcctgctttgagtattttagaggactgtgcctcgtagtaagaaaaaaatgaaactcagtttcttgaaccacaggatagagcctcctcaaatccaaatgctaccagctccagctcccaggatccagagagtttgcaagacagaggcgaagggaaggtcgcaacaacagttatctccaagatgctattcgttgaacccatcctggaggtttccagcttgccgacaaccaactcaacaaccaattcagccaccaaaataacagctaataccactgatgaacccaccacacaacccaccacagagcccaccacccaacccaccatccaacccacccaaccaactacccagctcccaacagattctcctacccagcccactactgggtccttctgcccaggacctgttactctctgctctgacttggagagtcattcaacagaggccgtgttgggggatgctttggtagatttctccctgaagctctaccacgccttctcagcaatgaagaaggtggagaccaacatggccttttccccattcagcatcgccagcctccttacccaggtcctgctcggtaagaccctgcttgaattctctccaggtcatttgttggacactcccataagagtcaccaatccagacacttacaaagccatgcctctgggaagaagctgtaaaaatgggctattatatattgggggtggggtagagggatgtatcttttcattcttgaacattccatcatttcacagtgatgtaataggcacgattgcttgtaaaactctgtgactatacaagaacatataaaataaggtcgcagccactaaccatgtttcatggcaaggagaggtgataagaaagatgaaattaggcgcagtggctcacgcctgtaatcccagcactttgggaggccaaggcgggtggatcacctgaggtcaggagttcaagaccagcctggccaacatggtgaaaccctgtctctactaaaaatacaaaaattatcagggagtggtggtgcatgcctgtaatcccagctacttgggcagctgaggcaggagaatcgcttgaacccaggaggtggaggttgcagtgagccgagaccgcaccattgcactacagtctgggtgacagagcgagactctgtctcaaaaaaaaaaaaaaattatcagagatagacctagagtagatgtggttagtactgccttctagctctgtgaccttgggcagatcactttaacctctctgagccttgagtcctcttgtgtaaaatagtgatgatgctatctacctcaaaagattaagaagcagaaagccaggccgggtgcggtggttcacacctgtaatcccagcattttaggaggccgaggcgggcagatcacgaggtcaggagttcgagaccagcctgactaacatggtgaaaccccgtctctactaaaaataaaaagaaattagctaggcatggtggtgcacacctgtaaccccagctactcaggaggctgaggcaggagaatcacttgaacacgggaggcagaggttgcagtgagccgaaatcatgccactgcactccagcctgggaagactgagcaagactctgtctcaaaaaaaaaaaagaagcagcctagtgtctgacttagtgggaggtcaaaaaaatgtaaatcctctgccatcttgagggattactgtcaagtcccatttggtaattaccctaggaatggcacaaacaaattactacaagcagtggggacagagctattactccccagagagaattctaaaaaggctacagaatctttcttggctgggcacggtgactcacacctataatcctggcactttgggaggccaaggcaggagttcaagaccagcctggccaacatgttgaaaccccatctctactaaaaatgcaaaaattagccaggcatagtgatgcatgcttattgtcccagctacttgggaggcagaggtgggaggattgcttgaacctggagattcaagtgagctgagattgcaccactgcattccagcctgggcaacaaagcaagactctgtctcaaaaaaaaaaaaaaaaaaaaaaaaagagagattgagagaacacttccagctcagatgatctgtgatcccctccaaagcagggaataccctccattccagcctggtccccaaccctcattcccaaggaaggcccccgactcatcctgcaagtatctttcatctctgccctttgttgcaggggctggggagaacaccaaaacaaacctggagagcatcctctcttaccccaaggacttcacctgtgtccaccaggccctgaagggcttcacgaccaaaggtgtcacctcagtctctcagatcttccacagcccaggtgagtgcccaggaatgggcagtgtctgcagaggagggtcctgagaggactctgaagggggacccagcgctggggaaagaaaggacagagggaatgttggagctacagtatcagggatggactgcagagcaggtgaagaccttggcaggagcattaggtcactccaggaactagactgttcttctaatgagaccttagacaagtctctggcattcatcaactgctttagaataaaaataaccgggcaggtacagtaaaatagtgatgatgctatctacctcaaaagattaagaagcagaaagccaggctgggcgtggtggctcacacctgtaatcccagcactttgggaggccgaggcaggtggatcacgaggtcaggggttcgagaccagcctgaccaacatggtgaaaccctgtctctactaaaaatacaaaaattagctgggcatggtggcgggcacctgtaatcccagctattcaggaggctgaggcaggagaattgcttgaacctgggaggcggaggttgcagtgagccgagatgacgccactgcactccagcctgggcgacagagcaagactccgtctcaaaaaaaaaaacaaaaacaaaacaaaaacaaaaaaaaaaacaaagaaggagaaagccgggccgggcatggtggctctcatctgtaagttcaaggagttgaaggtatgctaggactttgggaggccaaggccttcaagaccagcctgggcagcatggcgaaacctgtctccattaaaaaaaaaaaagttgggggtacggctgggcatggtggctcacacctgtaatcccagcactttgggaggctgaggtgggtggaacacctgaggtcaggagttcaagaccagcctggccaacatggcaaaaccctgtctctattaaaaacacaaaaattagcctggcatggtggcaggcgcctataatcccaactactcaggaggctgaggcaggagaatcgcttgaacccaagagagtgaaggttgcagtgagctgagatcatgccacttcactccagcctgagtgaaacagcaaaactctgtctcaaaaaaaaaaaaaggaagaaagaaaaaaggccaggcgcggtgactcacgcctgtaatcgcaacactttggcaggccgaggcaggcgattcacaaggtcaggagttcgagaccagtctggctaactaacatagtgaaactccgtctctactgaaaatacaagaaattaccctggcatggtggtgtgcacctgtaatcccagctactcaggaggctgaggcaggagaatcgcttgaacctgggaggcagaggctgcagtgagccgagatcgcgccactgcactccagcctggatgacagagcaagactctgtctcaaaaaaaaaaggccgggcgcggtggctcatgcctgtaatcccagcactttgggaggctgaggcgggcggaccacgaggtcagaagatcaagaccatcctggctaacaagatgaaaccctgtctctgccaaaaaaatacaaaacttagccgggcatggtggcaggcgcctgtggtcccaactacttgggaggctgaggcaggagaatggcatgaacccgggaggcggagcttgcagtgagccgagattgcgccactgcactccagcctgggcaacagagcgagacaccatctcaaaaaaaaaaaaaaaaaatggggcgggcgggccaggcgcggtgtctcacacctgtaatcccagcactttgggaggctgaggtgggcggatcacttgaggtcaggagttcaagaccagcctggccaacaccaggaaaccctgtctctgttaaaaatacaaaaattagccaggtgtggtggcacgcgcctgtagtcccagcaggagaataacttcaacctgggagacagaggttgcagtcagctgagatcgcaccactgcattccagcctgggtgacagaccgagactctgtctcaaaaaaaaaaaaaaaagaagaatacccatatgcattcattaatatatagggctagagggctagagagctatagacataaaatagacaaaaaatttttttgctcatttttgggtcaaaggagtcttgggactctaattcttttaatttttgtgttatgtgaatttgttatcatttacatgtattatgttattaagtaggtaataatgataatactaataataaacttacaaaacgatccaatgtagttgttttcagactttgttcctcggagccctaggactttgcaaagctgtttctggagtcatggtgggagtggggtgtggggagcctgagcagtggggaagggttcaccacttcctgtgagagggaaacggaccagctgggctctgagctccccacccagcctcagccagggtccattttatattgtgggcttcagacatgcctttgtttgaaagcagttctgctgctttaaaatgtttgataaccattgaactaatctacccacctccctttttaaaaaaaaaaggaaaacttttttttaagctgttttttttgttttttgtttttttttaaactgtaaaaacaatacttaggtctggctcagtgtgcctgtaattccaacactgagaggctgaggtaggaggattgcttgaggctagaatttcgagactagcctctgggcaacatagacagacctcatctctacaaaaaattttaaaaattatccgggtgtggtacgtgtctgtagttccagctatgaaggactgagacgggaggattgcttgagccaaggaattcgaagttagagtgagctatgtttatgcctctgtactctaggttgggtaacagagtaggaccctgtctctaaaaaaaaaaaaatttaatttaaattttaaaaactcacctatcaccccatcatctgaaaaacaccctctttcagatgtgggaaaaacatggctcagaggtgttcaagaaatgttgcatttatttattacttacaaagctgtaagtcagctttatccgctgtcttgctaggttggtgaaaaatacgtaacagcattcaatattagggcttctatccccatctagctgcacactggagctgtgccaagcaaggttcttggtcttatgttgtacttaggcatcagcaaagcctgggaaaatatcttttttttttttttgagacagaatctcgctctgtcgcccaggctggaatgcagtggcaccatctcagctcactgcaacctccgtctcccagattcaagtgattctcctgcctcagcctcccgaatagctgggattacaggctggtcttgaactcctggcctccagtgatccacccaccttggcctcccaaagtgctgcgattacaggtgtgagccaccatgcccagctggggaaaatatctttaatctacttagtcctagaaaaattatctttcaagtgctttttttttttttttcagtggactgaaggcttttgcagagcaaaagccaggaagttttgtcacaaacttccaccaaggccaggaagcagagtctattccgtgccaaaattaagggaagaaaagagggaaaatctaggcaaatggaatttaatatctcaaaaagattatcttgccgagccatagtcacatagcaagctgaggcagcggaggcttggggctacttctcttgttcttggttctgggtttaccttctttgggccttatttgccacatctgtaagaggagtgggctggaccgcgctccaccatgccgtattcactaagtgagcagatagaaccatagaaagcatgctcactctcaaatcgtgctcatggaaagaacgacgtgttcaggactcatgcctccctttctcaacatacccccagacctggccataagggacacctttgtgaatgcctctcggaccctgtacagcagcagccccagagtcctaagcaacaacagtgacgccaacttggagctcatcaacacctgggtggccaagaacaccaacaacaagatcagccggctgctagacagtctgccctccgatacccgccttgtcctcctcaatgctatctacctgagtggtaagggtgcccttagccagttagtcttcccattctgggtccttcttcccctcctggcttcaaagcccacttaaccccaagttctacaatcggatctcaatgtccctgcactactctttgctaacaaggcttttagctcctcttcatccttttcctacctgcattagagcaaccctcccacctcttccctctagccaagtggaagacaacatttgatcccaagaaaaccagaatggaaccctttcacttcaaaaactcagttataaaagtgcccatgatgaatagcaagaagtaccctgtggcccatttcattgaccaaactttgaaagccaaggtaagttcttaacctttccttctcctgtttgaaacctacttgagtctcctgactttttttctgctgtagtcccatcattttggggtacatgcttacaaattcatcacttctactccttccatctgtatttccaccctatcttttctccttctcctttctctagccttggccaaggcagacattgtatattttaggctggaaacaggattctcaagtttcttcatgcatctctactatattgaatggcaaaatgtgagtcgtgttcctattctacacatctgtttctttttccagtcaactcatcagaagactctggtggcttagcaagtcctgtgtgtatgtgggtacctgtgtacagcatacatatacatgtgtagacgtgtataagtatatccttgtatatgcatatatgtggtaagtgcatgtgtgcacatgagttaaatggcttaagtgcattagcagaaattgaacaatttagtttgatgagtagggagggagagaagacagaatatggagcccagaggatcccaactggcaagctatctcatccccagttaccagatatttccacctttttaggatggcaaaacacagacctatgagacagaaaacagtaagagacaatgtctcaatacctggctgagaaacaaaggctctgttcttggaacatgctaggcttggttccacattgggagctttccttagcttttgtttctgcctgtatccctcttcactcagatcctcacatagcttgttccttcttgtcatttgggtgtcagctcagaggtcaccttggtggagaagtcttctccccattaaagcagcctcctcctcaccctgtaatatcactcctgttttattatattcattacactcatcaccatctgaaattatgtcatttatttgcttatttgcctaggacattgtctgtctccctaagatactgtctctctacttgaatacaggaacctgtcttgtttccttctgtatctgtagtgcctagaacaatgcctcctatcataggtgctcattcagtgtttgctgaataaatgaatgaatgaaatagagggtgccaaagagagctactcagtaaaagtggctggaagacttcatagaggagggttttttttcgagacagggtctcactctgtcactcaagctgcagtgcattgacatgatctcagctcactgcaatctctgcctcccgagttcaagcagttctcctgcctcagcctcccaagtagctgggactacaggagcccgccaccacacctggctaatttttgtatttttagtagagacggggtttcaccatgttagccaagctggtctcgaactcctgacctcaagtgatccacaccctcagcctcccaaagggctgggattacaggcatgagccacagcacccagctgaggaggttatttttgaccattctttgctcagttatttatccactcatggacttatccacccatctatccatccctatctaatgtatttgaccattcatgactcatttagcagaaccaggacagcctgtataaggcacagaagagtgaatatatgtgacaggtccagagcattgttcaaattcaagatacgttgggggaggtataaatatgagatttttttcaaatcaattggaatggctatttaatcaaagccatagatgttaggtggaaagtaggaattaagaacttaacaagttaggtttaaatgtaactattcgaattataagaacaagtatttcctctctaaaaatgtttttaaagtttcacacaaaactctaaaccaaaaatcattgtaaaaatcccttgggagtagactgttgaaaccattgaggtgaggtgataggttaaggtgagcattctggacatataatatcaataataaatattcaaatacaaagcaggtataatatgaagagtaatttctatctccccaagccaatatgagttttgtttgtttgtttgtttttcttttgagataaagtctcattctgttgcccaggccggagtgcagtggcacaatcccagctctctgtaacctctgcctcccaggttcaagcgattctcctgccttagcctccctagtagctgggattataggcgcctgccaccactcccagctaatttttgtatttttagtagagatggggtttcaccatgttggccaggctggtcatgaactcctgacctcaagtgctcgtccgtcttcggcctcctaaagtgctggcattacaggcgtgagccactgcacccagcctgagttttttttttttttttaagccaaaggaggaggagtagttttgtgcacaaaagccactatttagagttccttaggttttaaacagataattaatttaatgtactaacaaatgcaaaattaaaattttacttatgccttttaattttaagctgaacttgctacattaagagtagggtgatttggctgggcgcagtggctcatgcctataatcccagcactttaggaggctgaggcaggtggatcacttgaagctaagagtttgagaccagcctggccaacatggtggaattctgtctctactaaaaatacaaaaattagccaggcatggtggcacatgtctgtaatcccagctactcaggatgctaaggcacagaatcacttgaacctgggaggcagaggttacagtgagccaaaatcgcgccactgcactccaacctgggcaacacagcaagactctgtctcaaaacacaaaaaaagaataggctgggtacagtggctcacgcctgtaatcccagcactttgggaggccgaggcaggtgaatcacctgaggtcaggagttcgagaccagcttggccaacattgtgaaaccccatctccattaaaaatacaaaaaataagccgggtgtgatggtgcacgcctgtaatcccagatacttgggaggctgggacagaagaatcgcttgaacccgggaggcgaaggttgcagtgagccgagatcatgccactgcattccagcctgagcgacagagtgagaccttgtctcagaaaaaaaaaaatagggtgatttttatataaaaacactctcatttgttcttgaattaattgccatattgaacagattaaactcctttaaaccattttttctatctacaaacataattagtattcccataagcattttaagctccctttaaaaatttaatatgctcgattttcttttttcttttatttatttatgtagttttcccagacagggtcttactctatcacccagtctggagtacagtgacacaatcctcacttactgtaacctcaagctccttgggatgaagcagtcctcccaccctagcctcttaagtagctgagattccaggcatgagccacctcacccagctgattttctttttaaacacatctaatacctgacaggtcgtaattacgactgtgcttggccatatcatcctaacacctaaagctcacttgtaaactgaaaattaaatttgaagggtgaattaacttctagccaacattccaatatcattctcacatttaatgaaattatcctacaactttgcttaaaagcataaaactagcatgtcagagtctcttaaaaattacaatcactattttaaataacaaacatacaggttaccctgaacttaacacctggttttaacatgatgaagttggtttcttttgtcattcttatactaaattctaaatcttcctggcacttaaggatatttacccaaggaagggggtgagatttaccggctcaggtacaccgaggttactggcttgaaaattcaagaccacagcatggtaaatttttcttcagagattcaaggttcatacataggacttgaagggcacatgctactcaaatgagtatatccaacttgagtgctacatcaacagggaccccatgtccactcttttcagtcgaaattggcttactatctacttcttctgggctattcagtttccgacaattgattgctttcagttaatttctttattgcccagttgaattctgcattcttctagattctttttgttccttcagcctcaatcataataccatttaatgacagtctcatatcctattagactagggtttctcagccttggcactattgacatattgggtcagataattctttgtcctgtgcattgtagaatttagcatcttccttagcttctactcactagaagccagtagcactgtgtgcacatcctccttgccccctgccagctatgacaaccaaaatgtctccagacattaccaaatgtccactgagaggcaaattcactctgagttgacaacccctgtattaaacccaggggccctgcacttcttacatacttttgtctggtcaccagttgaaagtccttcttcttttttttttctctttttgagatggagtctcgctctgtcaccaggctggagtgcagtggcatgatctcggctcactgcagcctccacctcccgggttcaagcaattctcctgcctcagcctcctgagtagctgggattacaggcacgtgccaccacccagctaatttttgtatttttagtagaggtggggtttcatcatggtggccaggatggtctcaatctcttgacctcatgatccgcccacctcggcctcccaaagtgctgggattacaggtgtgagccaccgtgcatgaccaaaagtccttctaatagcaaagtggaaaggtaggctgtgaacaatcttgaatgccatactaagatttgtacttattctcataggcagtgaagagccatcaatagtttttacagaggctgacctgataactctggcggttcaatgtgcatgctatatactatatgcacaacacattaggaaggaagggaacagcgctcagagaaatcaaatcacttgcccatattacatagctcgtcagtggtggagtcagggtataatcagaaactcatgctccttcctctacctctccccagcacagagttggatcagcactgttcacccagctggtatccccatttcatggtaaagcctggaagcttaggtctgactgatgcttgttgaaatacagactgtgggagcagactgcaggacagcattgtgacagagggtggggccaggagagagatgcggtaggaagactgttaaggtgcatctcttattttctaggtggggcagctgcagctctcccacaatctgagtttggtgatcctggtaccccagaacctgaaacatcgtcttgaagacatggaacaggctctcagcccttctgttttcaaggccatcatggagaaactggagatgtccaagttccagcccactctcctaacactaccccgcatcaaagtgacgaccagccaggatatgctctcaatcatggagaaattgggtgagctctggcagcttagggttactcccaggccatcagaggagaaaggggggatccctaagatgtagttagcattctctagagtattttttacatccataatctcagtttgtcctgcaaccctgcaagttagaggggtaggtgctattatcccattggatcattgtggaaatggaggctcagaagctttatgtgacttacccagagattccatgatttacccttgagctagtcagaggcaaaccagaacaccgacccaggtctccagctctcctgagttttttctatggttccttgtgacataggcagtggaacagtgggacaggtaaccgaggtgaattatggatgctccttccccagacacatttcaaaacagtcagccaccccgtggaatatgcaagaagctatctggaagtgcagatctggaggcttctgagtttacgagaggcaacagagactccattttcttttttttttttttttttgagacggagtcttgctctgtcacccaggacaggctggagtgcagtggtgcgatctctgctcactgcaagatccgcctcccagattcacgccatgccattctctcgcctcagcctcccgagtagctgggactacaggtgcccgccaccacgcctggctaattttgtttttgtatttttagtagagacggggtttcactgtgttaaccaggatggtcacaatctccggaccttgtgatccacctgcctcggcctcccaaagtgctgggattacaggcatgagtcaccgcgcccagcccagagactccattttctaacctttgtttttttgtttgtttgtttttgagacggagcctcactctgtcacccaggctggagcgcagtggcatgatcttgggtcactgcaacctccgcctcctgggttcaagtgattctcctacctcagcctcccaagtagctgggattacaggcacctaccaccacgcccagctaatttttttgtatttttagtagagatggggtttcaccatgttggtgaagctggtcttgaactcctgggctcaagtgatccacccacctcggcttcccaaagtgctgggattacaggtgtgagccactgtgcccagcctcattttctaacctttgatctcatgtccagccctgtcacttcatttcttgttagagaatttgaccgcctaacacatgattccatttccttgtatatgtcatctgtataggaagaaaacctcttttttattttcattcaacacttctggccaccaaacaggtgtgggagtgttttctaagcaattctccagttatctggggacaccaactgggtgtcctacaattgaatccaattctaacactctacctggaaataacatcagatcccgtgcagtttaagtgctccgccccagcaaatttccccccgtttccaatgtcagttacaagactgggttgtcacctgtgcatcagaccaaccagctataatttggagattcccacaactccctgctagggtttcatcatttgctagaatagctgacaaaactcaggagacacttacatttactggtttattatgtaaaggattaagtaaaggatacagatgaacagccagttgaagagatacatagggcaaaatctggaagggtcctgggcccagcagcatctatcctgtggagttctgtttgctaccttcctgacacatgtatgtgttcaccaaccagaaactctcagaaccctgtactttaggagaagtcatcatgtaggcatgattgattattacccaatctccagctcctctcttctccccagaggatggagagaggggctgaaagttccaagcttctaatcacacttggtctttctggtgaccagccccaatccaggagccagcaggagtagcctcattagcacaaaaggcattcctatgacccaggaaattccaagggatctagtagctctgtgtcaggaactgggatcggagaccaaatattagatggtctaatatttggagctaaagatgctcctatagcatattttcccattatttcacagcatcatggcattgcatataacctcattttttcatatatgacctatctctgatctattacctcacctccaaggtcctgggagataaggaggcaatgacatcatttttcagggttgttttagggatgaggggcaaggcctctcaccttgagagagagtggcagtgttgggcccactaatagaggatcccacgaactgccagagggtacagtatgtaatctggcaaacaagggaagaggaagagagcactgggactcaggatgaacccagagaattcaggacaaaggtctccatcagctgagggtatcatgctggcttctgactctgtttttctctggttttgccctagaattcttcgatttttcttatgaccttaacctgtgtgggctgacagaggacccagatcttcaggtttctgcgatgcagcaccagacagtgctggaactgacagagactggggtggaggcggctgcagcctccgccatctctgtggcccgcaccctgctggtctttgaagtgcagcagcccttcctcttcgtgctctgggaccagcagcacaagttccctgtcttcatggggcgagtatatgaccccagggcctgagacctgcaggatcaggttagggcgagcgctacctctccagcctcagctctcagttgcagccctgctgctgcctgcctggacttggcccctgccacctcctgcctcaggtgtccgctatccaccaaaagggctccctgagggtctgggcaagggacctgcttctattagcccttctccatggccctgccatgctctccaaaccactttttgcagctttctctagttcaagttcaccagactctataaataaaacctgacagaccatgactttctctgctttgcctttgtttttttattttttattttttattttttttaggcagggtctcaatctgtcacccaggctagagtacagtggtgagatcatggttcactgcagccttaacctcctgagctcaaacaatcctcccatctcagcctcctatgtaggtgggaccacatgggcttgccaccatgcccagctaatttttaaattttttgtaaagacagggtcttactatgttgcctaggctggtctccaactcctgggctcaagcaatcatcctaacacagcctcccgaagtgctgggattgtaggcacaccatacctctcctttgcctttgaatatcagctgcttcaatactaaaggacaagagcgcccatggttcctgtatcagccagctattgctgtatagtaagtcacgttaaacttagtggcttcaaacagcaaccctttgttattttatgtaagtttcagagttgactaggtgttttgctgatctgggctgaacctggctgatcttccctgggctcattcatacatctgtaaggtatagttgttgggttggttaggggatgactggtcttctgtggcctcagccatgacaccaggacaacttggctcttctacatgtcttgtatgtccttccaacaggctagtctgtaatggaaaagagtcaaacagccagtctctttttgtttaccattgtcctgcagccaaagcaaatcacaggaccaaacctagagttagactggaaaagcactacaaagtgacagggcaaagagacgttaattggggactattcatgcagtccatttctcacagcccctatcttgcttatttgtctgcaacaactctgacaacaataatgacagtagctaacgttgggaacataggcagtctgctaagagttttgcaggcatttaatcttcacaataaatttatatggtaaattcagagaggctaagtcttgttcaaagtcctgtagttaggaaatgatgaaactgagatttaatagcacctcttatgactcttttttttttgagacaaagtttctcttttgttgccaaggcttgagtataatagcacaatctcggctcactgtaacctctgcctcctgggttcaagtgattctcctgcctcagcctcccaagtagctgggattacaagcatgcactaccacacctggctaattttgtatttttagtagagacaggttttctttttttttttttttccgagatggagtcttgctttgtcggccaggctggagtgcagtggtgcaatcttggcttactcaacctccacctcccgggttcaagtagttctgcctcagcctcccaagtagctgggattacaggcgtgcaccaccaagcccagctaacttttgtatttttagtagagacggggtttcaccatgtggaccaggctggtctcaaactcctgactccaagtgatcttcccacctcagcctcccaaagtgctggcattacaggtgtgagccactgtgcccggcctagtgaaaacaatcttctttactcagtctaccagctcaaataccagtctcttcaggaaacaacctcacagacacacccagaaatgatatcttaccagttgtctgggcatcccttagcccagtaaaattgacacataaatttaaccaccccacaccttcccttctcagtttcccaaagtcaatctctcaggctgctgggaagaccccaaattcctgtctgggtgggtcccgctttgattcttatgtgaggaactgttgaaagcaaaggcaccccccaaattcaggaagattcccctctccttggggagatcctgacatgatgaaggtggtgctcagcaccaacctgaattgtgaaccaacaaagtcaggaggtggaaggtgattctgacccctgtgggggtcaaatctctttgacccttccaatcatgctgagcccggtaatgttcccgtttgtgaaatgatgaagccaaaactcagagaggttaagtaactatccaaaggtcagactgctgcaaatcgatcccacattatccaaattcaagtgtagtagataacttatttgggcaggcttatttcctttctgcccaaacttgactgtaacttaaatctgtgtcttcttactccctgcaccatgtgaccctacagagcttatcaaagtgtcttgcacttaaaaaaaaaaaaactatggaggctgggcatagtggctcatgcctataatgccagcactttgggagacggaggcaggcagatcacttgaggccagggttttgagaccagcctgggcaacatggcgaaaccctgtctctattaaaaaatacaaaaatgagccaggtgttgtggtgcatgcctgtaatcccagctactcgggaggctgaggcatgagaatcactttaacctggaaggcagaggttgcagtgaatccagattgtaccactccactccagcctgggtgacagagtgagagactgtctaaaaaaaaaaactatgaaatgaatgattaaatgaatgagttatcacatccaggtagagggaaagaggagatacctacccatctggaaagcatagaaaaatctggaaatgaagagaatttatttatttattttattttttgagacagagtcttgctctatcacccaggctggagtgcagcggcttgaacatggttcactgcagccttgacctcctgggctcaggtgatccttccacttcagcctcctgagtagcagggaccacaggtgtgcaccaccacacctggctacattttttgttttttataaagacagggtctcagctgggcacggtggctcatgcctgtaatgccagcactttgggaggccaaggcaggctgatcacctgagctcaggagttcgagaccagcctggcccacatggtgaaacctcgtctctattaaaaatacaaaaattaacaaggcgtggcagcaggcacatgtaatcccagctacttgcgggctgaggcaggagaatcacttgaacccaagaggtggaggttgcagtgagccgagatcatgccactgcactcctccagtctgggggatggagcaagacttcgccttggagaaaaaaaaaaaaagtctcactgtgttgcccaagctggtctggaactcctgggctcaagagatcctctagccttggcctcccaaaatgttgggattactggtgtgagccaccacacccaagataatttaaatattttctcttctgaagcttttcttataagagggcatgtgtcacttttttcgtttgtttaaaacaatgaacatttattttgctttgttttggttttttgtttttgtttttgttttgagacggagtcttgctctgtcttgcccaggctggagtacagtgacacaatctcggctcactgcagcctccgcctcctgggttcaaacaattctcctgtctcagcctcccgagtagctgggactacaggcttgtgccaccatgcctagctaatttttgtatctttagtagaaacgaggtttcactatgttggccaggctggtctcgaactcctgacctcaggtgacctgccctccttggccccccaaagtgccgggattacaggtataagccactgcacccagcctgaacatttattttgctaatgagtcattgacccagtgtgggcttggcaaatctagggtagcctcagttatgtacctgctacagtcagctgggggttagctgaaggtttgttgaggtttgatttcactgagcttgcataggctctttcacatgttttagactttggctgggatcaaccagatgaccaattctgatccaagtgatctctggtcttccaggaagctagtctggcttattcatacgaagtttgcaaaagtccaagaaagcaagcagaggcatgcatgcaaggcctcttgaatccgaagctaggaactactagaacatcacttctgcctcattctagcagccaaagcaagtcaccagaccagtttagattcaaggtaaggaaagaatctctacctgttaaagaaaagacctgcaaagtcattctgctaagggcattaatataacgaaatgtgaataattctggccacttttccagtataccatatgtggtcttacatagttgcaaacaactattagcaactttccccagcaacctgccactctgtttttccctaaagaatcaagggcttttgtcgagatcataataatattagaaacactttgttacatgaagtttcaagtcgtttgcatataaattgaatcttctgttgctatctctgtggcatatttaacaatctctggctcttccagctgcctgtgttgtagaataaattattataaatacagagctgcctgagtatttataataataaataaataaattatcttcatttccatttcccttgagaaagatggacagagggctatgcactcatagacacacacacacacacacacacacacacccttacaacccccacctttctgccctgccttgcaattctactctggggtagacaaaggcctgtatgtccacagatccattttcagtgatctgtttcctgtccccaactgtagacccctccacacgtggatttgtctggggaagaaccttaaggtgagattagggttccattgcaatgagtctttgctgccacttggtgtcattgttgaaggcttgtcctgcatagccccatggacacttgccttttcagggagatgtttttgctgttccagattcttttttttttttttttttgagacagaatctctctctgttgcccagactggagtgcaatggtgcgatcttggctcactgcaacctctgtttcccaggttgaagggattctcctgcctcagcttcctgagtagcaggaattataggcacccaccatgtgtccagctaatttttgtatttttagtagagatggggttttaccatgttggccaggctggtctcaaactcctgacctcaagtgatccacccatcttggcctcccaaagtgttagaattacaggtgtgagtcactgtgcctggccggttccagattcttaaacagctgatgtggggacttaaactttgattccaaagtttacactttacacttgttcagccactgtttctcaaagatcaatacctttagttctctctggatagcagaaggcttccaacatgagccataggctatgtcagaatcagcctcatccctatgaacccttaggacattgtcttgactcatggttgataaccacattagccatgtatctacctaacatgcattaaccatttgccatgctgtcaggcactgtgttaagaattttacatggattatgttatttcatttaagagagatcatgacttaagaaaaggatatgttactgaatatattagataattcaaaatttagataatttgatactaagttttccagaataataactgtaaaaggtagggagagaatcttcaaccattgtagaatttcttgtcttcaaactattgtttattttctaaatacaaaaatctctaatatttctcagagtaggcactcttaaattaactgcttggcatatcaggacagctatttgggctttttcatagtgtcttatcatatctaactttcattacaaagttattgattttggagggtgtttttagcactagt

SEQ ID NO: 3 - protein, 615 aa, Artificial Sequence
  Synthetic AAB59490.1 (FactorXII - AA)
MRALLLLGFLLVSLESTLSIPPWEAPKEHKYKAEEHTVVLTVTGEPCHFPFQYHRQLYHKCTHKGRPGPQPWCATTPNFDQDQRWGYCLEPKKVKDHCSKHSPCQKGGTCVNMPSGPHCLCPQHLTGNHCQKEKCFEPQLLRFFHKNEIWYRTEQAAVARCQCKGPDAHCQRLASQACRTNPCLHGGRCLEVEGHRLCHCPVGYTGPFCDVDTKASCYDGRGLSYRGLARTTLSGAPCQPWASEATYRNVTAEQARNWGLGGHAFCRNPDNDIRPWCFVLNRDRLSWEYCDLAQCQTPTQAAPPTPVSPRLHVPLMPAQPAPPKPQPTTRTPPQSQTPGALPAKREQPPSLTRNGPLSCGQRLRKSLSSMTRVVGGLVALRGAHPYIAALYWGHSFCAGSLIAPCWVLTAAHCLQDRPAPEDLTVVLGQERRNHSCEPCQTLAVRSYRLHEAFSPVSYQHDLALLRLQEDADGSCALLSPYVQPVCLPSGAARPSETTLCQVAGWGHQFEGAEEYASFLQEAQVPFLSLERCSAPDVHGSSILPGMLCAGFLEGGTDACQGDSGGPLVCEDQAAERRLTLQGIISWGSGCGDRNKPGVYTDVAYYLAWIREHTVS

SEQ ID NO: 4 - DNA, 1959 bp, Artificial Sequence
  Synthetic M11723.1 (FactorXII - Nucleotide)
ttggagtcaacactttcgattccaccttgggaagcccccaaggagcataagtacaaagctgaagagcacacagtcgttctcactgtcaccggggagccctgccacttccccttccagtaccaccggcagctgtaccacaaatgtacccacaagggccggccaggccctcagccctggtgtgctaccacccccaactttgatcaggaccagcgatggggatactgtttggagcccaagaaagtgaaagaccactgcagcaaacacagcccctgccagaaaggagggacctgtgtgaacatgccaagcggcccccactgtctctgtccacaacacctcactggaaaccactgccagaaagagaagtgctttgagcctcagcttctccggtttttccacaagaatgagatatggtatagaactgagcaagcagctgtggccagatgccagtgcaagggtcctgatgcccactgccagcggctggccagccaggcctgccgcaccaacccgtgcctccatgggggtcgctgcctagaggtggagggccaccgcctgtgccactgcccggtgggctacaccggacccttctgcgacgtggacaccaaggcaagctgctatgatggccgcgggctcagctaccgcggcctggccaggaccacgctctcgggtgcgccctgtcagccgtgggcctcggaggccacctaccggaacgtgactgccgagcaagcgcggaactggggactgggcggccacgccttctgccggaacccggacaacgacatccgcccgtggtgcttcgtgctgaaccgcgaccggctgagctgggagtactgcgacctggcacagtgccagaccccaacccaggcggcgcctccgaccccggtgtcccctaggcttcatgtcccactcatgcccgcgcagccggcaccgccgaagcctcagcccacgacccggaccccgtctcagtcccagaccccgggagccttgccggcgaagcgggagcagccgccttccctgaccaggaacggcccactgagctgcgggcagcggctccgcaagagtctgtcttcgatgacccgcgtcgttggcgggctggtggcgctacgcggggcgcacccctacatcgccgcgctgtactggggccacagtttctgcgccggcagcctcatcgccccctgctgggtgctgacggccgctcactgcctgcaggaccggcccgcacccgaggatctgacggtggtgctcggccaggaacgccgtaaccacagctgtgagccgtgccagacgttggccgtgcgctcctaccgcttgcacgaggccttctcgcccgtcagctaccagcacgacctggctctgttgcgccttcaggaggatgcggacggcagctgcgcgctcctgtcgccttacgttcagccggtgtgcctgccaagcggcgccgcgcgaccctccgagaccacgctctgccaggtggccggctggggccaccagttcgagggggcggaggaatatgccagcttcctgcaggaggcgcaggtaccgttcctctccctggagcgctgctcagccccggacgtgcacggatcctccatcctccccggcatgctctgcgcagggttcctcgagggcggcaccgatgcgtgccagggtgattccggaggcccgctggtgtgtgaggaccaagctgcagagcgccggctcaccctgcaaggcatcatcagctggggatcgggctgtggtgaccgcaacaagccaggcgtctacaccgatgtggcctactacctggcctggatccgggagcacaccgtttcctgattgctcagggactcatctttccctccttggtgattccgcagtgagagagtggctggggcatggaaggcaagattgtgtcccattcccccagtgcggccagctccgcgccaggatggcgcaggaactcaataaagtgctttgaaaatgctg